European Patent Application EP 4 279 509 A1, published November 22, 2023. Title: GARP Protein Antibody and Application Thereof. Applicant: SHANGHAI JEMINCARE PHARMACEUTICAL CO., LTD.; JIANGXI JEMINCARE GROUP CO., LTD. The sequence listing filed with the application follows.

SEQUENCE LISTING (54 sequences)

SEQ ID NO: 1 - protein, 123 aa, Artificial Sequence
  8H2D7B3 VH;1907hz0 VH
QVQLQQSGAELVRPGSSVKLSCKASGYTLSNYWMYWVKQRPIQGLEWIGSIAPSDSETHYNQKFKDRATVTVDKSSRIVYMQLSSLTSEDSAVYFCARGGFGYGSSHWYFDVWGTGTTVTVSS

SEQ ID NO: 2 - protein, 7 aa, Artificial Sequence
  8H2D7B3 HCDR1;1907hz0 HCDR1;JYB1907hz18 HCDR1
GYTLSNY

SEQ ID NO: 3 - protein, 6 aa, Artificial Sequence
  8H2D7B3 HCDR2;JYB1907hz0 HCDR2;JYB1907hz18 HCDR2
APSDSE

SEQ ID NO: 4 - protein, 14 aa, Artificial Sequence
  8H2D7B3 HCDR3;JYB1907hz0 HCDR3;JYB1907hz18 HCDR3
GGFGYGSSHWYFDV

SEQ ID NO: 5 - protein, 25 aa, Artificial Sequence
  8H2D7B3 H-FR1;1907hz0 H-FR1
QVQLQQSGAELVRPGSSVKLSCKAS

SEQ ID NO: 6 - protein, 19 aa, Artificial Sequence
  8H2D7B3 H-FR2;1907hz0 H-FR2
WMYWVKQRPIQGLEWIGSI

SEQ ID NO: 7 - protein, 41 aa, Artificial Sequence
  8H2D7B3 H-FR3;1907hz0 H-FR3
THYNQKFKDRATVTVDKSSRIVYMQLSSLTSEDSAVYFCAR

SEQ ID NO: 8 - protein, 11 aa, Artificial Sequence
  8H2D7B3 H-FR4;1907hz0 H-FR4
WGTGTTVTVSS

SEQ ID NO: 9 - protein, 107 aa, Artificial Sequence
  8H2D7B3 VL;1907hz0 VL
DIQMTQSSAYLSVSLGGRVTITCKASDHINKWLAWYQQKPGNAPRLLISGATSLETGIPSRFSGSGSGKDYTLSITGLQTEDVATYYCQQYWTTPYTFGGGTKLEIK

SEQ ID NO: 10 - protein, 11 aa, Artificial Sequence
  8H2D7B3 LCDR1;1907Hz0 LCDR1
KASDHINKWLA

SEQ ID NO: 11 - protein, 7 aa, Artificial Sequence
  8H2D7B3 LCDR2;1907Hz0 LCDR2
GATSLET

SEQ ID NO: 12 - protein, 9 aa, Artificial Sequence
  8H2D7B3 LCDR3;1907Hz0 VL LCDR3;JYB1907hz18 LCDR3
QQYWTTPYT

SEQ ID NO: 13 - protein, 23 aa, Artificial Sequence
  8H2D7B3 L-FR1;1907hz0 L-FR1
DIQMTQSSAYLSVSLGGRVTITC

SEQ ID NO: 14 - protein, 15 aa, Artificial Sequence
  8H2D7B3 L-FR2;1907hz0 L-FR2;1907hz18 L-FR2
WYQQKPGNAPRLLIS

SEQ ID NO: 15 - protein, 32 aa, Artificial Sequence
  8H2D7B3 L-FR3; 1907Hz0 L-FR3
GIPSRFSGSGSGKDYTLSITGLQTEDVATYYC

SEQ ID NO: 16 - protein, 10 aa, Artificial Sequence
  8H2D7B3 L-FR4;1907Hz0 L-FR4
FGGGTKLEIK

SEQ ID NO: 17 - protein, 327 aa, Artificial Sequence
  heavy chain constant region
ASTKGPSVFPLAPCSRSTSESTAALGCLVKDYFPEPVTVSWNSGALTSGVHTFPAVLQSSGLYSLSSVVTVPSSSLGTKTYTCNVDHKPSNTKVDKRVESKYGPPCPPCPAPEFLGGPSVFLFPPKPKDTLMISRTPEVTCVVVDVSQEDPEVQFNWYVDGVEVHNAKTKPREEQFNSTYRVVSVLTVLHQDWLNGKEYKCKVSNKGLPSSIEKTISKAKGQPREPQVYTLPPSQEEMTKNQVSLTCLVKGFYPSDIAVEWESNGQPENNYKTTPPVLDSDGSFFLYSRLTVDKSRWQEGNVFSCSVMHEALHNHYTQKSLSLSLGK

SEQ ID NO: 18 - protein, 107 aa, Artificial Sequence [sequence omitted]

SEQ ID NO: 19 - protein, 450 aa, Artificial Sequence
  1907hz0 heavy chain
QVQLQQSGAELVRPGSSVKLSCKASGYTLSNYWMYWVKQRPIQGLEWIGSIAPSDSETHYNQKFKDRATVTVDKSSRIVYMQLSSLTSEDSAVYFCARGGFGYGSSHWYFDVWGTGTTVTVSSASTKGPSVFPLAPCSRSTSESTAALGCLVKDYFPEPVTVSWNSGALTSGVHTFPAVLQSSGLYSLSSVVTVPSSSLGTKTYTCNVDHKPSNTKVDKRVESKYGPPCPPCPAPEFLGGPSVFLFPPKPKDTLMISRTPEVTCVVVDVSQEDPEVQFNWYVDGVEVHNAKTKPREEQFNSTYRVVSVLTVLHQDWLNGKEYKCKVSNKGLPSSIEKTISKAKGQPREPQVYTLPPSQEEMTKNQVSLTCLVKGFYPSDIAVEWESNGQPENNYKTTPPVLDSDGSFFLYSRLTVDKSRWQEGNVFSCSVMHEALHNHYTQKSLSLSLGK

SEQ ID NO: 20 - protein, 214 aa, Artificial Sequence
  1907Hz0 light chain
DIQMTQSSAYLSVSLGGRVTITCKASDHINKWLAWYQQKPGNAPRLLISGATSLETGIPSRFSGSGSGKDYTLSITGLQTEDVATYYCQQYWTTPYTFGGGTKLEIKRTVAAPSVFIFPPSDEQLKSGTASVVCLLNNFYPREAKVQWKVDNALQSGNSQESVTEQDSKDSTYSLSSTLTLSKADYEKHKVYACEVTHQGLSSPVTKSFNRGEC

SEQ ID NO: 21 - protein, 123 aa, Artificial Sequence
  JYB1907hz18 VH
QVQLVQSGAEVKKPGASVKVSCKASGYTLSNYWMYWVRQAPGQGLEWIGSIAPSDSETHYNQKFQGRVTVTVDKSTRIVYMELSSLRSEDTAVYFCARGGFGYGSSHWYFDVWGQGTMVTVSS

SEQ ID NO: 22 - protein, 25 aa, Artificial Sequence [sequence omitted]

SEQ ID NO: 23 - protein, 19 aa, Artificial Sequence
  1907Hz18 H-FR2
WMYWVRQAPGQGLEWIGSI

SEQ ID NO: 24 - protein, 41 aa, Artificial Sequence
  1907Hz18 H-FR3
THYNQKFQGRVTVTVDKSTRIVYMELSSLRSEDTAVYFCAR

SEQ ID NO: 25 - protein, 11 aa, Artificial Sequence
  1907Hz18 H-FR4
WGQGTMVTVSS

SEQ ID NO: 26 - protein, 107 aa, Artificial Sequence
  JYB1907hz18 VL
DIQMTQSPSTLSASVGDRVTITCRASDHINKWLAWYQQKPGNAPRLLISGATSLESGVPSRFSGSGSGKDYTLTISSLQPDDFATYYCQQYWTTPYTFGQGTKLEIK

SEQ ID NO: 27 - protein, 11 aa, Artificial Sequence
  JYB1907hz18 LCDR1
RASDHINKWLA

SEQ ID NO: 28 - protein, 7 aa, Artificial Sequence
  JYB1907hz18 LCDR2
GATSLES

SEQ ID NO: 29 - protein, 23 aa, Artificial Sequence
  1907Hz18 L-FR1
DIQMTQSPSTLSASVGDRVTITC

SEQ ID NO: 30 - protein, 32 aa, Artificial Sequence
  1907Hz18 L-FR3
GVPSRFSGSGSGKDYTLTISSLQPDDFATYYC

SEQ ID NO: 31 - protein, 10 aa, Artificial Sequence
  1907Hz18 L-FR4
FGQGTKLEIK

SEQ ID NO: 32 - protein, 450 aa, Artificial Sequence
  JYB1907hz18 heavy chain
QVQLVQSGAEVKKPGASVKVSCKASGYTLSNYWMYWVRQAPGQGLEWIGSIAPSDSETHYNQKFQGRVTVTVDKSTRIVYMELSSLRSEDTAVYFCARGGFGYGSSHWYFDVWGQGTMVTVSSASTKGPSVFPLAPCSRSTSESTAALGCLVKDYFPEPVTVSWNSGALTSGVHTFPAVLQSSGLYSLSSVVTVPSSSLGTKTYTCNVDHKPSNTKVDKRVESKYGPPCPPCPAPEFLGGPSVFLFPPKPKDTLMISRTPEVTCVVVDVSQEDPEVQFNWYVDGVEVHNAKTKPREEQFNSTYRVVSVLTVLHQDWLNGKEYKCKVSNKGLPSSIEKTISKAKGQPREPQVYTLPPSQEEMTKNQVSLTCLVKGFYPSDIAVEWESNGQPENNYKTTPPVLDSDGSFFLYSRLTVDKSRWQEGNVFSCSVMHEALHNHYTQKSLSLSLGK

SEQ ID NO: 33 - protein, 214 aa, Artificial Sequence
  JYB1907hz18 light chain
DIQMTQSPSTLSASVGDRVTITCRASDHINKWLAWYQQKPGNAPRLLISGATSLESGVPSRFSGSGSGKDYTLTISSLQPDDFATYYCQQYWTTPYTFGQGTKLEIKRTVAAPSVFIFPPSDEQLKSGTASVVCLLNNFYPREAKVQWKVDNALQSGNSQESVTEQDSKDSTYSLSSTLTLSKADYEKHKVYACEVTHQGLSSPVTKSFNRGEC

SEQ ID NO: 34 - protein, 118 aa, Artificial Sequence [sequence omitted]

SEQ ID NO: 35 - protein, 10 aa, Artificial Sequence
  Anti-PD-L1 antibody HCDR1
GFTFSDSWIH

SEQ ID NO: 36 - protein, 18 aa, Artificial Sequence
  Anti-PD-L1 antibody HCDR2
AWISPYGGSTYYADSVKG

SEQ ID NO: 37 - protein, 9 aa, Artificial Sequence
  Anti-PD-L1 antibody HCDR3
RHWPGGFDY

SEQ ID NO: 38 - protein, 107 aa, Artificial Sequence [sequence omitted]

SEQ ID NO: 39 - protein, 11 aa, Artificial Sequence
  Anti-PD-L1 antibody LCDR1
RASQDVSTAVA

SEQ ID NO: 40 - protein, 7 aa, Artificial Sequence
  Anti-PD-L1 antibody LCDR2
SASFLYS

SEQ ID NO: 41 - protein, 9 aa, Artificial Sequence
  Anti-PD-L1 antibody LCDR3
QQYLYHPAT

SEQ ID NO: 42 - protein, 448 aa, Artificial Sequence
  Anti-PD-L1 antibody  heavy chain
EVQLVESGGGLVQPGGSLRLSCAASGFTFSDSWIHWVRQAPGKGLEWVAWISPYGGSTYYADSVKGRFTISADTSKNTAYLQMNSLRAEDTAVYYCARRHWPGGFDYWGQGTLVTVSSASTKGPSVFPLAPSSKSTSGGTAALGCLVKDYFPEPVTVSWNSGALTSGVHTFPAVLQSSGLYSLSSVVTVPSSSLGTQTYICNVNHKPSNTKVDKKVEPKSCDKTHTCPPCPAPELLGGPSVFLFPPKPKDTLMISRTPEVTCVVVDVSHEDPEVKFNWYVDGVEVHNAKTKPREEQYASTYRVVSVLTVLHQDWLNGKEYKCKVSNKALPAPIEKTISKAKGQPREPQVYTLPPSREEMTKNQVSLTCLVKGFYPSDIAVEWESNGQPENNYKTTPPVLDSDGSFFLYSKLTVDKSRWQQGNVFSCSVMHEALHNHYTQKSLSLSPGK

SEQ ID NO: 43 - protein, 214 aa, Artificial Sequence
  Anti-PD-L1 antibody  light chain
DIQMTQSPSSLSASVGDRVTITCRASQDVSTAVAWYQQKPGKAPKLLIYSASFLYSGVPSRFSGSGSGTDFTLTISSLQPEDFATYYCQQYLYHPATFGQGTKVEIKRTVAAPSVFIFPPSDEQLKSGTASVVCLLNNFYPREAKVQWKVDNALQSGNSQESVTEQDSKDSTYSLSSTLTLSKADYEKHKVYACEVTHQGLSSPVTKSFNRGEC

SEQ ID NO: 44 - protein, 11 aa, Artificial Sequence
  8H2D7B3 LCDR1; 1907Hz0 VL LCDR1; JYB1907hz18 LCDR1 formula
  misc_feature (1)..(1): Xaa = Lys or Arg
XASDHINKWLA

SEQ ID NO: 45 - protein, 7 aa, Artificial Sequence
  8H2D7B3 LCDR2; 1907Hz0 VL LCDR2; JYB1907hz18 LCDR2 formula
  misc_feature (7)..(7): Xaa = Ser or Thr
GATSLEX

SEQ ID NO: 46 - protein, 25 aa, Artificial Sequence
  8H2D7B3 H-FR1; 1907Hz0 H-FR1; 1907Hz18 H-FR1 formula
  misc_feature (5)..(5): Xaa = Gln or Val
  misc_feature (11)..(11): Xaa = Leu or Val
  misc_feature (12)..(12): Xaa = Lys or Val
  misc_feature (13)..(13): Xaa = Lys or Arg
  misc_feature (16)..(16): Xaa = Ala or Ser
  misc_feature (20)..(20): Xaa = Leu or Val
QVQLXQSGAEXXXPGXSVKXSCKAS

SEQ ID NO: 47 - protein, 19 aa, Artificial Sequence
  8H2D7B3 H-FR2; 1907Hz0 H-FR2; 1907Hz18 H-FR2 formula
  misc_feature (6)..(6): Xaa = Lys or Arg
  misc_feature (8)..(8): Xaa = Ala or Arg
  misc_feature (10)..(10): Xaa = Gly or Ile
WMYWVXQXPXQGLEWIGSI

SEQ ID NO: 48 - protein, 41 aa, Artificial Sequence
  8H2D7B3 H-FR3; 1907Hz0 H-FR3; 1907Hz18 H-FR3 formula
  misc_feature (8)..(8): Xaa = Lys or Gln
  misc_feature (9)..(9): Xaa = Asp or Gly
  misc_feature (11)..(11): Xaa = Ala or Val
  misc_feature (19)..(19): Xaa = Ser or Thr
  misc_feature (25)..(25): Xaa = Glu or Gln
  misc_feature (30)..(30): Xaa = Arg or Thr
  misc_feature (34)..(34): Xaa = Ser or Thr
THYNQKFXXRXTVTVDKSXRIVYMXLSSLXSEDXAVYFCAR

SEQ ID NO: 49 - protein, 11 aa, Artificial Sequence
  8H2D7B3 H-FR4; 1907Hz0 H-FR4; 1907Hz18 H-FR4 formula
  misc_feature (3)..(3): Xaa = Gln or Thr
  misc_feature (6)..(6): Xaa = Met or Thr
WGXGTXVTVSS

SEQ ID NO: 50 - protein, 123 aa, Artificial Sequence
  8H2D7B3 VH; 1907Hz0 VH; JYB1907hz18 VH formula
  misc_feature (5)..(5): Xaa = Gln or Val
  misc_feature (11)..(11): Xaa = Leu or Val
  misc_feature (12)..(12): Xaa = Lys or Val
  misc_feature (13)..(13): Xaa = Lys or Arg
  misc_feature (16)..(16): Xaa = Ala or Ser
  misc_feature (20)..(20): Xaa = Leu or Val
  misc_feature (38)..(38): Xaa = Lys or Arg
  misc_feature (40)..(40): Xaa = Ala or Arg
  misc_feature (42)..(42): Xaa = Gly or Ile
  misc_feature (65)..(65): Xaa = Lys or Gln
  misc_feature (66)..(66): Xaa = Asp or Gly
  misc_feature (68)..(68): Xaa = Ala or Val
  misc_feature (76)..(76): Xaa = Ser or Thr
  misc_feature (82)..(82): Xaa = Glu or Gln
  misc_feature (87)..(87): Xaa = Arg or Thr
  misc_feature (91)..(91): Xaa = Ser or Thr
  misc_feature (115)..(115): Xaa = Gln or Thr
  misc_feature (118)..(118): Xaa = Met or Thr
QVQLXQSGAEXXXPGXSVKXSCKASGYTLSNYWMYWVXQXPXQGLEWIGSIAPSDSETHYNQKFXXRXTVTVDKSXRIVYMXLSSLXSEDXAVYFCARGGFGYGSSHWYFDVWGXGTXVTVSS

SEQ ID NO: 51 - protein, 107 aa, Artificial Sequence
  8H2D7B3 VL; 1907Hz0 VL; JYB1907hz18 VL formula
  misc_feature (8)..(8): Xaa = Pro or Ser
  misc_feature (9)..(9): Xaa = Ala or Ser
  misc_feature (10)..(10): Xaa = Thr or Tyr
  misc_feature (13)..(13): Xaa = Ala or Val
  misc_feature (15)..(15): Xaa = Leu or Val
  misc_feature (17)..(17): Xaa = Asp or Gly
  misc_feature (24)..(24): Xaa = Lys or Arg
  misc_feature (56)..(56): Xaa = Ser or Thr
  misc_feature (58)..(58): Xaa = Ile or Val
  misc_feature (74)..(74): Xaa = Ser or Thr
  misc_feature (76)..(76): Xaa = Ser or Thr
  misc_feature (77)..(77): Xaa = Gly or Ser
  misc_feature (80)..(80): Xaa = Pro or Thr
  misc_feature (81)..(81): Xaa = Asp or Glu
  misc_feature (83)..(83): Xaa = Phe or Val
  misc_feature (100)..(100): Xaa = Gly or Gln
DIQMTQSXXXLSXSXGXRVTITCXASDHINKWLAWYQQKPGNAPRLLISGATSLEXGXPSRFSGSGSGKDYTLXIXXLQXXDXATYYCQQYWTTPYTFGXGTKLEIK

SEQ ID NO: 52 - protein, 23 aa, Artificial Sequence
  8H2D7B3 L-FR1; 1907Hz0 L-FR1; 1907Hz18 L-FR1 formula
  misc_feature (8)..(8): Xaa = Pro or Ser
  misc_feature (9)..(9): Xaa = Ala or Ser
  misc_feature (10)..(10): Xaa = Thr or Tyr
  misc_feature (13)..(13): Xaa = Ala or Val
  misc_feature (15)..(15): Xaa = Leu or Val
  misc_feature (17)..(17): Xaa = Asp or Gly
DIQMTQSXXXLSXSXGXRVTITC

SEQ ID NO: 53 - protein, 32 aa, Artificial Sequence
  8H2D7B3 L-FR3; 1907Hz0 L-FR3; 1907Hz18 L-FR3 formula
  misc_feature (2)..(2): Xaa = Ile or Val
  misc_feature (18)..(18): Xaa = Ser or Thr
  misc_feature (20)..(20): Xaa = Ser or Thr
  misc_feature (21)..(21): Xaa = Gly or Ser
  misc_feature (24)..(24): Xaa = Pro or Thr
  misc_feature (25)..(25): Xaa = Asp or Glu
  misc_feature (27)..(27): Xaa = Phe or Val
GXPSRFSGSGSGKDYTLXIXXLQXXDXATYYC

SEQ ID NO: 54 - protein, 10 aa, Artificial Sequence
  8H2D7B3 L-FR4; 1907Hz0 L-FR4; 1907Hz18 L-FR4 formula
  misc_feature (3)..(3): Xaa = Gly or Gln
FGXGTKLEIK